European Patent Application EP 4 775 594 A1, published July 15, 2026. Title: Bispecific antibodies that bind CD3 and the ganglioside NGcGM3. Applicant: CENTRO DE INMUNOLOGIA MOLECULAR. Application CU 2023-0043, filed September 8, 2023. The sequence listing filed with the application follows.

SEQUENCE LISTING (16 sequences)

SEQ ID NO: 1 - protein, 329 aa, synthetic construct
ASTKGPSVFPLAPSSKSTSGGTAALGCLVKDYFPEPVTVSWNSGALTSGVHTFPAVLQSSGLYSLSSVVTVPSSSLGTQTYICNVNHKPSNTKVDKKVEPKSCDKTHTCPPCPAPPVAGPSVFLFPPKPKDTLMISRTPEVTCVVVGVSHEDPEVKFNWYVDGVEVHNAKTKPREEQYNSTYRVVSVLTVLHQDWLNGKEYKCKVSNKQLPSPIEKTISKAKGQPREPQVYTLPPSRDELTKNQVSLTCLVKGFYPSDIAVEWESNGQPENNYKTTPPVLDSDGSFFLYSKLTVDKSRWQQGNVFSCSVMHEALHNHYTQKSLSLSPGK

SEQ ID NO: 2 - protein, 330 aa, synthetic construct
ASTKGPSVFPLAPSSKSTSGGTAALGCLVKDYFPEPVTVSWNSGALTSGVHTFPAVLQSSGLYSLSSVVTVPSSSLGTQTYICNVNHKPSNTKVDKKVEPKSCDKTHTCPPCPAPELLGGPSVFLFPPKPKDTLMISRTPEVTCVVVDVSHEDPEVKFNWYVDGVEVHNAKTKPREEQYXSTYRVVSVLTVLHQDWLNGKEYKCKVSNKALPAPIEKTISKAKGQPREPQVYTLPPSRDELTKNQVSLTCLVKGFYPSDIAVEWESNGQPENNYKTTPPVLDSDGSFFLYSKLTVDKSRWQQGNVFSCSVMHEALHNHYTQKSLSLSPGK

SEQ ID NO: 3 - protein, 326 aa, synthetic construct
ASTKGPSVFPLAPCSRSTSESTAALGCLVKDYFPEPVTVSWNSGALTSGVHTFPAVLQSSGLYSLSSVVTVPSSNFGTQTYTCNVDHKPSNTKVDKTVERKCCVECPPCPAPPVAGPSVFLFPPKPKDTLMISRTPEVTCVVVDVSHEDPEVQFNWYVDGVEVHNAKTKPREEQFNSTFRVVSVLTVVHQDWLNGKEYKCKVSNKGLPAPIEKTISKTKGQPREPQVYTLPPSREEMTKNQVSLTCLVKGFYPSDISVEWESNGQPENNYKTTPPMLDSDGSFFLYSKLTVDKSRWQQGNVFSCSVMHEALHNHYTQKSLSLSPGK

SEQ ID NO: 4 - protein, 327 aa, synthetic construct
ASTKGPSVFPLAPCSRSTSESTAALGCLVKDYFPEPVTVSWNSGALTSGVHTFPAVLQSSGLYSLSSVVTVPSSSLGTKTYTCNVDHKPSNTKVDKRVESKYGPPCPSCPAPEFLGGPSVFLFPPKPKDTLMISRTPEVTCVVVDVSQEDPEVQFNWYVDGVEVHNAKTKPREEQFNSTYRVVSVLTVLHQDWLNGKEYKCKVSNKGLPSSIEKTISKAKGQPREPQVYTLPPSQEEMTKNQVSLTCLVKGFYPSDIAVEWESNGQPENNYKTTPPVLDSDGSFFLYSRLTVDKSRWQEGNVFSCSVMHEALHNHYTQKSLSLSLGK

SEQ ID NO: 5 - protein, 244 aa, synthetic construct
DIQMTQSPSSLSASVGDRVTITCRASQDIRNYLNWYQQKPGKAPKLLIYYTSRLESGVPSRFSGSGSGTDYTLTISSLQPEDFATYYCQQGNTLPWTFGQGTKVEIKGGGGSGGGGSGGGGSEVQLVESGGGLVQPGGSLRLSCAASGYSFTGYTMNWVRQAPGKGLEWVALINPYKGVSTYNQKFKDRFTISVDKSKNTAYLQMNSLRAEDTAVYYCARSGYYGDSDWYFDVWGQGTLVTVSS

SEQ ID NO: 6 - protein, 240 aa, synthetic construct
DIQMTQSPSSLSASVGDRVTITCSASSVSYMNWYQQTPGKAPKRWIYDTSKLASGVPSRFSGSGSGTDYTFTISSLQPEDIATYYCOOWSSNPFTFGQGTKLQITRGGGGSGGGGSGGGGSQVQLVQSGGGVVQPGRSLRLSCKASGYTFTRYTMHWVRQAPGKGLEWIGYINPSRGYTNYNOKVKDRFTISRDNSKNTAFLQMDSLRPEDTGVYFCARYYDDHYCLDYWGQGTPVTVSS

SEQ ID NO: 7 - protein, 240 aa, synthetic construct
DIKLQQSGAELARPGASVKMSCKTSGYTFTRYTMHWVKQRPGQGLEWIGYINPSRGYTNYNQKFKDKATLTTDKSSSTAYMQLSSLTSEDSAVYYCARYYDDHYCLDYWGQGTTLTVSSGGGGSGGGGSGGGGSDIQLTQSPAIMSASPGEKVTMTCRASSSVSYMNWYQQKSGTSPKRWIYDTSKVASGVPYRFSGSGSGTSYSLTISSMEAEDAATYYCQQWSSNPLTFGAGTKLELK

SEQ ID NO: 8 - protein, 107 aa, synthetic construct [sequence omitted]

SEQ ID NO: 9 - protein, 106 aa, synthetic construct
GQPKANPTVTLFPPSSEELQANKATLVCLISDFYPGAVTVAWKADGSPVKAGVETTKPSKQSNNKYAASSYLSLTPEQWKSHRSYSCQVTHEGSTVEKTVAPTECS

SEQ ID NO: 10 - protein, 125 aa, synthetic construct
QVQLQQSGNELAKPGASMKMSCRASGYSFTSYWIHWLKQRPDQGLEWIGYIDPATAYTESNQKFKDKAILTADRSSNTAFMYLNSLTSEDSAVYYCARESPRLRRGIYYYAMDYWGQGTTVTVSS

SEQ ID NO: 11 - protein, 109 aa, synthetic construct
DLVLTQSPATLSVTPGDSVSFSCRASQSISNNLHWYQQRTHESPRLLIKYASQSISGIPSRFSGSGSGTDFTLSIISVETEDFGMYFCQQSNRWPLTFGAGTKLELKRA

SEQ ID NO: 12 - protein, 107 aa, synthetic construct
DIQMTQTPSSLSASLGDRVTISCRASQDISNYLNWYQQKPDGTVKLLIYYTSRLHSGVPSRFSGSGSGTDYSLTISNLEQEDIATYFCQQGNTLPPTFGAGTKLELK

SEQ ID NO: 13 - protein, 107 aa, Synthetic construct
SSELTQDPAVSVALGQTRITCQGDSLRSYYASWYQQKPGQAPVLVIYGKNNRPSGIPDRFSGSSSGNTASLTITGAQAEDEADYYCNSRDSSGNHVVFGGGTKLTVL

SEQ ID NO: 14 - protein, 107 aa, synthetic construct
DLVLTQSPATLSVTPGDSVSFSCRASQSISNNLHWYQQKPGQSPRLLIKYASQSISGVPSRFSGSGSGTDFTLSIISVETEDFGMYFCQQSNRWPLTFGAGTKLELK

SEQ ID NO: 15 - protein, 125 aa, synthetic construct
QVQLVQSGAEVVKPGASMKMSCRASGYSFTSYWIHWLKQRPDQGLEWVGYIDPATAYTESNQKFKDKAILTADRSSNTAFMYLNSLTSEDSAVYYCARESPRLRRGIYYYAMDYWGQGTTVTVSS

SEQ ID NO: 16 - protein, 239 aa, synthetic construct
EVQLVESGGGLVQPGKSLKLSCEASGFTFSGYGMHWVRQAPGRGLESVAYITSSSINIKYADAVKGRFTVSRDNAKNLLFLQMNILKSEDTAMYYCARFDWDKNYWGQGTMVTVSSGGGGSGGGGSGGGGSDIQMTQSPSSLPASLGDRVTINCQASQDISNYLNWYQQKPGKAPKLLIYYTNKLADGVPSRFSGSGSGRDSSFTISSLESEDIGSYYCQQYYNYPWTFGPGTKLEIKR